European Patent Application EP 4 674 868 A1, published January 7, 2026. Title: FAP/4-1BB/CD40 BINDING MOLECULE AND MEDICINAL USE THEREOF. Applicant: JIANGSU HENGRUI PHARMACEUTICALS CO., LTD. The sequence listing filed with the application follows.

SEQUENCE LISTING (80 sequences)

SEQ ID NO: 1 - protein, 125 aa, synthetic construct
  source 1..125: note = Ab10 VH
QVQLQQSGVEVKKPGASVTVSCRASGYSFADHFIHWVRQAPGQGFQWMGWINPNRGVTHHAQDFQGRVAMTRDMSTDTVYMELTSLRSDDTAVYYCARDASLTARPYYFYGFDVWGQGTLVTVSS

SEQ ID NO: 2 - protein, 107 aa, synthetic construct
  source 1..107: note = Ab10 VL
DIQMTQSPSSVSASVGDRVTITCRASQGISSWLAWYQQKPGKAPKLLIYAASSLQSGVPSRFSGSGSGTDFTLTISSLQPEDFATYYCQQANSFPPAFGQGTKVEIK

SEQ ID NO: 3 - protein, 5 aa, synthetic construct
  source 1..5: note = CDR
DHFIH

SEQ ID NO: 4 - protein, 17 aa, synthetic construct
  source 1..17: note = CDR
WINPNRGVTHHAQDFQG

SEQ ID NO: 5 - protein, 16 aa, synthetic construct
  source 1..16: note = CDR
DASLTARPYYFYGFDV

SEQ ID NO: 6 - protein, 11 aa, synthetic construct
  source 1..11: note = CDR
RASQGISSWLA

SEQ ID NO: 7 - protein, 7 aa, synthetic construct
  source 1..7: note = CDR
AASSLQS

SEQ ID NO: 8 - protein, 9 aa, synthetic construct
  source 1..9: note = CDR
QQANSFPPA

SEQ ID NO: 9 - protein, 455 aa, synthetic construct
  source 1..455: note = Ab10 HC
QVQLQQSGVEVKKPGASVTVSCRASGYSFADHFIHWVRQAPGQGFQWMGWINPNRGVTHHAQDFQGRVAMTRDMSTDTVYMELTSLRSDDTAVYYCARDASLTARPYYFYGFDVWGQGTLVTVSSASTKGPSVFPLAPSSKSTSGGTAALGCLVKDYFPEPVTVSWNSGALTSGVHTFPAVLQSSGLYSLSSVVTVPSSSLGTQTYICNVNHKPSNTKVDKKVEPKSCDKTHTCPPCPAPEAAGGPSVFLFPPKPKDTLMISRTPEVTCVVVDVSHEDPEVKFNWYVDGVEVHNAKTKPREEQYNSTYRVVSVLTVLHQDWLNGKEYKCKVSNKALPAPIEKTISKAKGQPREPQVYTLPPSRDELTKNQVSLTCLVKGFYPSDIAVEWESNGQPENNYKTTPPVLDSDGSFFLYSKLTVDKSRWQQGNVFSCSVMHEALHNHYTQKSLSLSPGK

SEQ ID NO: 10 - protein, 214 aa, synthetic construct
  source 1..214: note = Ab10 LC
DIQMTQSPSSVSASVGDRVTITCRASQGISSWLAWYQQKPGKAPKLLIYAASSLQSGVPSRFSGSGSGTDFTLTISSLQPEDFATYYCQQANSFPPAFGQGTKVEIKRTVAAPSVFIFPPSDEQLKSGTASVVCLLNNFYPREAKVQWKVDNALQSGNSQESVTEQDSKDSTYSLSSTLTLSKADYEKHKVYACEVTHQGLSSPVTKSFNRGEC

SEQ ID NO: 11 - protein, 117 aa, synthetic construct
  source 1..117: note = A297
QVQLVESGGGMVEPGGSLRLSCAASGFTFSRYGMKWVRQAPGKGPEWVSTINSHGDTTYYADSVKGRFTISRDNAQNTVYLQMNSLKPEDTALYYCLRIDYSDYSSRGQGTQVTVSS

SEQ ID NO: 12 - protein, 5 aa, synthetic construct
  source 1..5: note = CDR
RYGMK

SEQ ID NO: 13 - protein, 17 aa, synthetic construct
  source 1..17: note = CDR
TINSHGDTTYYADSVKG

SEQ ID NO: 14 - protein, 8 aa, synthetic construct
  source 1..8: note = CDR
IDYSDYSS

SEQ ID NO: 15 - protein, 117 aa, synthetic construct
  source 1..117: note = A297V3
EVQLVESGGGLVQPGGSLRLSCAASGFTFSRYGMKWVRQAPGKGLEWVSTINSHGDTTYYADSVKGRFTISRDNAKNSLYLQMNSLRAEDTAVYYCLRIDYSDYSSRGQGTLVTVSS

SEQ ID NO: 16 - protein, 232 aa, synthetic construct
  source 1..232: note = IgG1-Fc
EPKSADKTHTCPPCPAPELLGGPSVFLFPPKPKDTLMISRTPEVTCVVVDVEHEDPEVKFNWYVDGVEVHNAKTKPREEQYNSTYRVVSVLTVLHQDWLNGKEYKCKVSSKAFPAPIEKTISKAKGQPREPQVYTLPPSRDELTKNQVSLTCLVKGFYPSDIAVEWESNGQPENNYKTTPPVLDSDGSFFLYSKLTVDKSRWQQGNVFSCSVMHEALHNHYTQKSLSLSPGK

SEQ ID NO: 17 - protein, 163 aa, synthetic construct
  source 1..163: note = 4-1BB
LQDPCSNCPAGTFCDNNRNQICSPCPPNSFSSAGGQRTCDICRQCKGVFRTRKECSSTSNAECDCTPGFHCLGAGCSMCEQDCKQGQELTKKGCKDCCFGTFNDQKRGICRPWTNCSLDGKSVLVNGTKERDVVCGPSPADLSPGASSVTPPAPAREPGHSPQ

SEQ ID NO: 18 - protein, 124 aa, synthetic construct
  source 1..124: note = C5
QVQLVESGGGLVQPGGSLRLSCSASGFTFSSYAMSWVRQAPGKGLEWVSDINSGGESTFYEDSVKGRFTISRDNAKNTLYLQMNSLKPEDTAVYYCAKHPLTFTIATMNDYDYWGQGTQVTVSS

SEQ ID NO: 19 - protein, 5 aa, synthetic construct
  source 1..5: note = CDR
SYAMS

SEQ ID NO: 20 - protein, 17 aa, synthetic construct
  source 1..17: note = CDR
DINSGGESTFYEDSVKG

SEQ ID NO: 21 - protein, 15 aa, synthetic construct
  source 1..15: note = CDR
HPLTFTIATMNDYDY

SEQ ID NO: 22 - protein, 356 aa, synthetic construct
  source 1..356: note = C5-Fc
QVQLVESGGGLVQPGGSLRLSCSASGFTFSSYAMSWVRQAPGKGLEWVSDINSGGESTFYEDSVKGRFTISRDNAKNTLYLQMNSLKPEDTAVYYCAKHPLTFTIATMNDYDYWGQGTQVTVSSEPKSADKTHTCPPCPAPELLGGPSVFLFPPKPKDTLMISRTPEVTCVVVDVEHEDPEVKFNWYVDGVEVHNAKTKPREEQYNSTYRVVSVLTVLHQDWLNGKEYKCKVSNKAFPAPIEKTISKAKGQPREPQVYTLPPSREEMTKNQVSLTCLVKGFYPSDIAVEWESNGQPENNYKTTPPVLDSDGSFFLYSKLTVDKSRWQQGNVFSCSVMHEALHNHYTQKSLSLSPGA

SEQ ID NO: 23 - protein, 124 aa, synthetic construct
  source 1..124: note = C5_V1
QVQLVESGGGLVQPGGSLRLSCSASGFTFSSYAMSWVRQAPGKGLEWVSDINSGGESTFYEDSVKGRFTISRDNAKNTLYLQMNSLRAEDTAVYYCARHPLTFTIATMNDYDYWGQGTLVTVSS

SEQ ID NO: 24 - protein, 124 aa, synthetic construct
  source 1..124: note = C5_V2
QVQLVESGGGLVQPGGSLRLSCSASGFTFSSYAMSWVRQAPGKGLEWVSDINSGGESTFYEDSVKGRFTISRDNAKNTLYLQMNSLRAEDTAVYYCAKHPLTFTIATMNDYDYWGQGTLVTVSS

SEQ ID NO: 25 - protein, 124 aa, synthetic construct
  source 1..124: note = C5_V3
QVQLVESGGGLVQPGGSLRLSCSASGFTFSSYAMSWVRQAPGKGLEWVSDINSGGESTFYEDSVKGRFTISRDNAKNTLYLQMNSLKPEDTAVYYCAKHPLTFTIATMNDYDYWGQGTLVTVSS

SEQ ID NO: 26 - protein, 124 aa, synthetic construct
  source 1..124: note = C5_V2-YTI
QVQLVESGGGLVQPGGSLRLSCSASGFTFSSYAMSWVRQAPGKGLEWVSDINSGGESTFYEDSVKGRFTISRDNAKNTLYLQMNSLRAEDTAVYYCAKHPLTYTIATMNDYDYWGQGTLVTVSS

SEQ ID NO: 27 - protein, 15 aa, synthetic construct
  source 1..15: note = CDR
HPLTYTIATMNDYDY

SEQ ID NO: 28 - protein, 124 aa, synthetic construct
  source 1..124: note = C5_V2-YTIQ
QVQLVESGGGLVQPGGSLRLSCSASGFTFSSYAMSWVRQAPGKGLEWVSDINSGGQSTFYADSVKGRFTISRDNAKNTLYLQMNSLRAEDTAVYYCAKHPLTYTIATMNDYDYWGQGTQVTVSS

SEQ ID NO: 29 - protein, 17 aa, synthetic construct
  source 1..17: note = CDR
DINSGGQSTFYADSVKG

SEQ ID NO: 30 - protein, 17 aa, synthetic construct
  source 1..17: note = CDR
  VARIANT 7: note = X is E or Q
  VARIANT 12: note = X is E or A
DINSGGXSTFYXDSVKG

SEQ ID NO: 31 - protein, 15 aa, synthetic construct
  source 1..15: note = CDR
  VARIANT 5: note = X is F or Y
HPLTXTIATMNDYDY

SEQ ID NO: 32 - protein, 118 aa, synthetic construct
  source 1..118: note = A297V3_AA
EVQLVESGGGLVQPGGSLRLSCAASGFTFSRYGMKWVRQAPGKGLEWVSTINSHGDTTYYADSVKGRFTISRDNAKNSLYLQMNSLRAEDTAVYYCLRIDYSDYSSRGQGTLVTVSAA

SEQ ID NO: 33 - protein, 125 aa, synthetic construct
  source 1..125: note = C5_V2-YTI_AA
QVQLVESGGGLVQPGGSLRLSCSASGFTFSSYAMSWVRQAPGKGLEWVSDINSGGESTFYEDSVKGRFTISRDNAKNTLYLQMNSLRAEDTAVYYCAKHPLTYTIATMNDYDYWGQGTLVTVSAA

SEQ ID NO: 34 - protein, 716 aa, synthetic construct
  source 1..716: note = B977703
QVQLQQSGVEVKKPGASVTVSCRASGYSFADHFIHWVRQAPGQGFQWMGWINPNRGVTHHAQDFQGRVAMTRDMSTDTVYMELTSLRSDDTAVYYCARDASLTARPYYFYGFDVWGQGTLVTVSSASTKGPSVFPLAPSSKSTSGGTAALGCLVKDYFPEPVTVSWNSGALTSGVHTFPAVLQSSGLYSLSSVVTVPSSSLGTQTYICNVNHKPSNTKVDKKVEPKSCDKTHTCPPCPAPEAAGGPSVFLFPPKPKDTLMISRTPEVTCVVVDVSHEDPEVKFNWYVDGVEVHNAKTKPREEQYNSTYRVVSVLTVLHQDWLNGKEYKCKVSNKALPAPIEKTISKAKGQPREPQVYTLPPSRDELTKNQVSLTCLVKGFYPSDIAVEWESNGQPENNYKTTPPVLDSDGSFFLYSKLTVDKSRWQQGNVFSCSVMHEALHNHYTQKSLSLSPGKGGGGSGGGGSQVQLVESGGGLVQPGGSLRLSCSASGFTFSSYAMSWVRQAPGKGLEWVSDINSGGESTFYEDSVKGRFTISRDNAKNTLYLQMNSLRAEDTAVYYCAKHPLTYTIATMNDYDYWGQGTLVTVSSGGGGSGGGGSEVQLVESGGGLVQPGGSLRLSCAASGFTFSRYGMKWVRQAPGKGLEWVSTINSHGDTTYYADSVKGRFTISRDNAKNSLYLQMNSLRAEDTAVYYCLRIDYSDYSSRGQGTLVTVSS

SEQ ID NO: 35 - protein, 214 aa, synthetic construct; identical to SEQ ID NO: 10
  source 1..214: note = B977703

SEQ ID NO: 36 - protein, 589 aa, synthetic construct
  source 1..589: note = B977704
QVQLQQSGVEVKKPGASVTVSCRASGYSFADHFIHWVRQAPGQGFQWMGWINPNRGVTHHAQDFQGRVAMTRDMSTDTVYMELTSLRSDDTAVYYCARDASLTARPYYFYGFDVWGQGTLVTVSSASTKGPSVFPLAPSSKSTSGGTAALGCLVKDYFPEPVTVSWNSGALTSGVHTFPAVLQSSGLYSLSSVVTVPSSSLGTQTYICNVNHKPSNTKVDKKVEPKSCDKTHTCPPCPAPEAAGGPSVFLFPPKPKDTLMISRTPEVTCVVVDVSHEDPEVKFNWYVDGVEVHNAKTKPREEQYNSTYRVVSVLTVLHQDWLNGKEYKCKVSNKALPAPIEKTISKAKGQPREPQVYTLPPSRDELTKNQVSLTCLVKGFYPSDIAVEWESNGQPENNYKTTPPVLDSDGSFFLYSKLTVDKSRWQQGNVFSCSVMHEALHNHYTQKSLSLSPGKGGGGSGGGGSQVQLVESGGGLVQPGGSLRLSCSASGFTFSSYAMSWVRQAPGKGLEWVSDINSGGESTFYEDSVKGRFTISRDNAKNTLYLQMNSLRAEDTAVYYCAKHPLTYTIATMNDYDYWGQGTLVTVSS

SEQ ID NO: 37 - protein, 341 aa, synthetic construct
  source 1..341: note = B977704
DIQMTQSPSSVSASVGDRVTITCRASQGISSWLAWYQQKPGKAPKLLIYAASSLQSGVPSRFSGSGSGTDFTLTISSLQPEDFATYYCQQANSFPPAFGQGTKVEIKRTVAAPSVFIFPPSDEQLKSGTASVVCLLNNFYPREAKVQWKVDNALQSGNSQESVTEQDSKDSTYSLSSTLTLSKADYEKHKVYACEVTHQGLSSPVTKSFNRGECGGGGSGGGGSEVQLVESGGGLVQPGGSLRLSCAASGFTFSRYGMKWVRQAPGKGLEWVSTINSHGDTTYYADSVKGRFTISRDNAKNSLYLQMNSLRAEDTAVYYCLRIDYSDYSSRGQGTLVTVSS

SEQ ID NO: 38 - protein, 723 aa, synthetic construct
  source 1..723: note = B977707
QVQLQQSGVEVKKPGASVTVSCRASGYSFADHFIHWVRQAPGQGFQWMGWINPNRGVTHHAQDFQGRVAMTRDMSTDTVYMELTSLRSDDTAVYYCARDASLTARPYYFYGFDVWGQGTLVTVSSASTKGPSVFPLAPSSKSTSGGTAALGCLVKDYFPEPVTVSWNSGALTSGVHTFPAVLQSSGLYSLSSVVTVPSSSLGTQTYICNVNHKPSNTKVDKKVEPKSCDKTHTCPPCPAPEAAGGPSVFLFPPKPKDTLMISRTPEVTCVVVDVSHEDPEVKFNWYVDGVEVHNAKTKPREEQYNSTYRVVSVLTVLHQDWLNGKEYKCKVSNKALPAPIEKTISKAKGQPREPQVYTLPPSRDELTKNQVSLTCLVKGFYPSDIAVEWESNGQPENNYKTTPPVLDSDGSFFLYSKLTVDKSRWQQGNVFSCSVMHEALHNHYTQKSLSLSPGKGGGGSGGGGSQVQLVESGGGLVQPGGSLRLSCSASGFTFSSYAMSWVRQAPGKGLEWVSDINSGGESTFYEDSVKGRFTISRDNAKNTLYLQMNSLRAEDTAVYYCAKHPLTYTIATMNDYDYWGQGTLVTVSSGGGGSGGGGSQVQLVESGGGLVQPGGSLRLSCSASGFTFSSYAMSWVRQAPGKGLEWVSDINSGGESTFYEDSVKGRFTISRDNAKNTLYLQMNSLRAEDTAVYYCAKHPLTYTIATMNDYDYWGQGTLVTVSS

SEQ ID NO: 39 - protein, 341 aa, synthetic construct; identical to SEQ ID NO: 37
  source 1..341: note = B977707

SEQ ID NO: 40 - protein, 716 aa, synthetic construct
  source 1..716: note = B785502
QVQLQQSGVEVKKPGASVTVSCRASGYSFADHFIHWVRQAPGQGFQWMGWINPNRGVTHHAQDFQGRVAMTRDMSTDTVYMELTSLRSDDTAVYYCARDASLTARPYYFYGFDVWGQGTLVTVSSASTKGPSVFPLAPSSKSTSGGTAALGCLVKDYFPEPVTVSWNSGALTSGVHTFPAVLQSSGLYSLSSVVTVPSSSLGTQTYICNVNHKPSNTKVDKKVEPKSCDKTHTCPPCPAPEAAGGPSVFLFPPKPKDTLMISRTPEVTCVVVDVSHEDPEVKFNWYVDGVEVHNAKTKPREEQYNSTYRVVSVLTVLHQDWLNGKEYKCKVSNKALPAPIEKTISKAKGQPREPQVYTLPPSRDELTKNQVSLTCLVKGFYPSDIAVEWESNGQPENNYKTTPPVLDSDGSFFLYSKLTVDKSRWQQGNVFSCSVMHEALHNHYTQKSLSLSPGKGGGGSGGGGSEVQLVESGGGLVQPGGSLRLSCAASGFTFSRYGMKWVRQAPGKGLEWVSTINSHGDTTYYADSVKGRFTISRDNAKNSLYLQMNSLRAEDTAVYYCLRIDYSDYSSRGQGTLVTVSSGGGGSGGGGSQVQLVESGGGLVQPGGSLRLSCSASGFTFSSYAMSWVRQAPGKGLEWVSDINSGGESTFYEDSVKGRFTISRDNAKNTLYLQMNSLRAEDTAVYYCAKHPLTFTIATMNDYDYWGQGTLVTVSS

SEQ ID NO: 41 - protein, 214 aa, synthetic construct; identical to SEQ ID NO: 10
  source 1..214: note = B785502

SEQ ID NO: 42 - protein, 582 aa, synthetic construct
  source 1..582: note = B785503
QVQLQQSGVEVKKPGASVTVSCRASGYSFADHFIHWVRQAPGQGFQWMGWINPNRGVTHHAQDFQGRVAMTRDMSTDTVYMELTSLRSDDTAVYYCARDASLTARPYYFYGFDVWGQGTLVTVSSASTKGPSVFPLAPSSKSTSGGTAALGCLVKDYFPEPVTVSWNSGALTSGVHTFPAVLQSSGLYSLSSVVTVPSSSLGTQTYICNVNHKPSNTKVDKKVEPKSCDKTHTCPPCPAPEAAGGPSVFLFPPKPKDTLMISRTPEVTCVVVDVSHEDPEVKFNWYVDGVEVHNAKTKPREEQYNSTYRVVSVLTVLHQDWLNGKEYKCKVSNKALPAPIEKTISKAKGQPREPQVYTLPPSRDELTKNQVSLTCLVKGFYPSDIAVEWESNGQPENNYKTTPPVLDSDGSFFLYSKLTVDKSRWQQGNVFSCSVMHEALHNHYTQKSLSLSPGKGGGGSGGGGSEVQLVESGGGLVQPGGSLRLSCAASGFTFSRYGMKWVRQAPGKGLEWVSTINSHGDTTYYADSVKGRFTISRDNAKNSLYLQMNSLRAEDTAVYYCLRIDYSDYSSRGQGTLVTVSS

SEQ ID NO: 43 - protein, 348 aa, synthetic construct
  source 1..348: note = B785503
DIQMTQSPSSVSASVGDRVTITCRASQGISSWLAWYQQKPGKAPKLLIYAASSLQSGVPSRFSGSGSGTDFTLTISSLQPEDFATYYCQQANSFPPAFGQGTKVEIKRTVAAPSVFIFPPSDEQLKSGTASVVCLLNNFYPREAKVQWKVDNALQSGNSQESVTEQDSKDSTYSLSSTLTLSKADYEKHKVYACEVTHQGLSSPVTKSFNRGECGGGGSGGGGSQVQLVESGGGLVQPGGSLRLSCSASGFTFSSYAMSWVRQAPGKGLEWVSDINSGGESTFYEDSVKGRFTISRDNAKNTLYLQMNSLRAEDTAVYYCAKHPLTFTIATMNDYDYWGQGTLVTVSS

SEQ ID NO: 44 - protein, 483 aa, synthetic construct
  source 1..483: note = B785511
QVQLVESGGGLVQPGGSLRLSCSASGFTFSSYAMSWVRQAPGKGLEWVSDINSGGESTFYEDSVKGRFTISRDNAKNTLYLQMNSLRAEDTAVYYCAKHPLTFTIATMNDYDYWGQGTLVTVSSEPKSADKTHTCPPCPAPEAAGGPSVFLFPPKPKDTLMISRTPEVTCVVVDVSHEDPEVKFNWYVDGVEVHNAKTKPREEQYNSTYRVVSVLTVLHQDWLNGKEYKCKVSNKALPAPIEKTISKAKGQPREPQVYTLPPSRDELTKNQVSLTCLVKGFYPSDIAVEWESNGQPENNYKTTPPVLDSDGSFFLYSKLTVDKSRWQQGNVFSCSVMHEALHNHYTQKSLSLSPGKGGGGSGGGGSEVQLVESGGGLVQPGGSLRLSCAASGFTFSRYGMKWVRQAPGKGLEWVSTINSHGDTTYYADSVKGRFTISRDNAKNSLYLQMNSLRAEDTAVYYCLRIDYSDYSSRGQGTLVTVSS

SEQ ID NO: 45 - protein, 717 aa, synthetic construct
  source 1..717: note = B21326101
QVQLQQSGVEVKKPGASVTVSCRASGYSFADHFIHWVRQAPGQGFQWMGWINPNRGVTHHAQDFQGRVAMTRDMSTDTVYMELTSLRSDDTAVYYCARDASLTARPYYFYGFDVWGQGTLVTVSSASTKGPSVFPLAPSSKSTSGGTAALGCLVKDYFPEPVTVSWNSGALTSGVHTFPAVLQSSGLYSLSSVVTVPSSSLGTQTYICNVNHKPSNTKVDKKVEPKSCDKTHTCPPCPAPEAAGGPSVFLFPPKPKDTLMISRTPEVTCVVVDVSHEDPEVKFNWYVDGVEVHNAKTKPREEQYNSTYRVVSVLTVLHQDWLNGKEYKCKVSNKALPAPIEKTISKAKGQPREPQVYTLPPSRDELTKNQVSLTCLVKGFYPSDIAVEWESNGQPENNYKTTPPVLDSDGSFFLYSKLTVDKSRWQQGNVFSCSVMHEALHNHYTQKSLSLSPGKGGGGSGGGGSQVQLVESGGGLVQPGGSLRLSCSASGFTFSSYAMSWVRQAPGKGLEWVSDINSGGESTFYEDSVKGRFTISRDNAKNTLYLQMNSLRAEDTAVYYCAKHPLTYTIATMNDYDYWGQGTLVTVSSGGGGSGGGGSEVQLVESGGGLVQPGGSLRLSCAASGFTFSRYGMKWVRQAPGKGLEWVSTINSHGDTTYYADSVKGRFTISRDNAKNSLYLQMNSLRAEDTAVYYCLRIDYSDYSSRGQGTLVTVSAA

SEQ ID NO: 46 - protein, 214 aa, synthetic construct; identical to SEQ ID NO: 10
  source 1..214: note = B21326101

SEQ ID NO: 47 - protein, 590 aa, synthetic construct
  source 1..590: note = B21326102
QVQLQQSGVEVKKPGASVTVSCRASGYSFADHFIHWVRQAPGQGFQWMGWINPNRGVTHHAQDFQGRVAMTRDMSTDTVYMELTSLRSDDTAVYYCARDASLTARPYYFYGFDVWGQGTLVTVSSASTKGPSVFPLAPSSKSTSGGTAALGCLVKDYFPEPVTVSWNSGALTSGVHTFPAVLQSSGLYSLSSVVTVPSSSLGTQTYICNVNHKPSNTKVDKKVEPKSCDKTHTCPPCPAPEAAGGPSVFLFPPKPKDTLMISRTPEVTCVVVDVSHEDPEVKFNWYVDGVEVHNAKTKPREEQYNSTYRVVSVLTVLHQDWLNGKEYKCKVSNKALPAPIEKTISKAKGQPREPQVYTLPPSRDELTKNQVSLTCLVKGFYPSDIAVEWESNGQPENNYKTTPPVLDSDGSFFLYSKLTVDKSRWQQGNVFSCSVMHEALHNHYTQKSLSLSPGKGGGGSGGGGSQVQLVESGGGLVQPGGSLRLSCSASGFTFSSYAMSWVRQAPGKGLEWVSDINSGGESTFYEDSVKGRFTISRDNAKNTLYLQMNSLRAEDTAVYYCAKHPLTYTIATMNDYDYWGQGTLVTVSAA

SEQ ID NO: 48 - protein, 342 aa, synthetic construct
  source 1..342: note = B21326102
DIQMTQSPSSVSASVGDRVTITCRASQGISSWLAWYQQKPGKAPKLLIYAASSLQSGVPSRFSGSGSGTDFTLTISSLQPEDFATYYCQQANSFPPAFGQGTKVEIKRTVAAPSVFIFPPSDEQLKSGTASVVCLLNNFYPREAKVQWKVDNALQSGNSQESVTEQDSKDSTYSLSSTLTLSKADYEKHKVYACEVTHQGLSSPVTKSFNRGECGGGGSGGGGSEVQLVESGGGLVQPGGSLRLSCAASGFTFSRYGMKWVRQAPGKGLEWVSTINSHGDTTYYADSVKGRFTISRDNAKNSLYLQMNSLRAEDTAVYYCLRIDYSDYSSRGQGTLVTVSAA

SEQ ID NO: 49 - protein, 717 aa, synthetic construct
  source 1..717: note = B21546901
QVQLQQSGVEVKKPGASVTVSCRASGYSFADHFIHWVRQAPGQGFQWMGWINPNRGVTHHAQDFQGRVAMTRDMSTDTVYMELTSLRSDDTAVYYCARDASLTARPYYFYGFDVWGQGTLVTVSSASTKGPSVFPLAPSSKSTSGGTAALGCLVKDYFPEPVTVSWNSGALTSGVHTFPAVLQSSGLYSLSSVVTVPSSSLGTQTYICNVNHKPSNTKVDKKVEPKSCDKTHTCPPCPAPEAAGGPSVFLFPPKPKDTLMISRTPEVTCVVVDVSHEDPEVKFNWYVDGVEVHNAKTKPREEQYNSTYRVVSVLTVLHQDWLNGKEYKCKVSNKALPAPIEKTISKAKGQPREPQVYTLPPSRDELTKNQVSLTCLVKGFYPSDIAVEWESNGQPENNYKTTPPVLDSDGSFFLYSKLTVDKSRWQQGNVFSCSVMHEALHNHYTQKSLSLSPGKGGGGSGGGGSQVQLVESGGGLVQPGGSLRLSCSASGFTFSSYAMSWVRQAPGKGLEWVSDINSGGQSTFYADSVKGRFTISRDNAKNTLYLQMNSLRAEDTAVYYCAKHPLTYTIATMNDYDYWGQGTQVTVSSGGGGSGGGGSEVQLVESGGGLVQPGGSLRLSCAASGFTFSRYGMKWVRQAPGKGLEWVSTINSHGDTTYYADSVKGRFTISRDNAKNSLYLQMNSLRAEDTAVYYCLRIDYSDYSSRGQGTQVTVSAA

SEQ ID NO: 50 - protein, 214 aa, synthetic construct; identical to SEQ ID NO: 10
  source 1..214: note = B21546901

SEQ ID NO: 51 - protein, 710 aa, synthetic construct
  source 1..710: note = RO7122290
REGPELSPDDPAGLLDLRQGMFAQLVAQNVLLIDGPLSWYSDPGLAGVSLTGGLSYKEDTKELVVAKAGVYYVFFQLELRRVVAGEGSGSVSLALHLQPLRSAAGAAALALTVDLPPASSEARNSAFGFQGRLLHLSAGQRLGVHLHTEARARHAWQLTQGATVLGLFRVTPEIPAGLGGGGSGGGGSREGPELSPDDPAGLLDLRQGMFAQLVAQNVLLIDGPLSWYSDPGLAGVSLTGGLSYKEDTKELVVAKAGVYYVFFQLELRRVVAGEGSGSVSLALHLQPLRSAAGAAALALTVDLPPASSEARNSAFGFQGRLLHLSAGQRLGVHLHTEARARHAWQLTQGATVLGLFRVTPEIPAGLGGGGSGGGGSRTVAAPSVFIFPPSDRKLKSGTASVVCLLNNFYPREAKVQWKVDNALQSGNSQESVTEQDSKDSTYSLSSTLTLSKADYEKHKVYACEVTHQGLSSPVTKSFNRGECDKTHTCPPCPAPEAAGGPSVFLFPPKPKDTLMISRTPEVTCVVVDVSHEDPEVKFNWYVDGVEVHNAKTKPREEQYNSTYRVVSVLTVLHQDWLNGKEYKCKVSNKALGAPIEKTISKAKGQPREPQVYTLPPCRDELTKNQVSLWCLVKGFYPSDIAVEWESNGQPENNYKTTPPVLDSDGSFFLYSKLTVDKSRWQQGNVFSCSVMHEALHNHYTQKSLSLSPGK

SEQ ID NO: 52 - protein, 447 aa, synthetic construct
  source 1..447: note = RO7122290
EVQLLESGGGLVQPGGSLRLSCAASGFTFSSYAMSWVRQAPGKGLEWVSAIIGSGASTYYADSVKGRFTISRDNSKNTLYLQMNSLRAEDTAVYYCAKGWFGGFNYWGQGTLVTVSSASTKGPSVFPLAPSSKSTSGGTAALGCLVKDYFPEPVTVSWNSGALTSGVHTFPAVLQSSGLYSLSSVVTVPSSSLGTQTYICNVNHKPSNTKVDKKVEPKSCDKTHTCPPCPAPEAAGGPSVFLFPPKPKDTLMISRTPEVTCVVVDVSHEDPEVKFNWYVDGVEVHNAKTKPREEQYNSTYRVVSVLTVLHQDWLNGKEYKCKVSNKALGAPIEKTISKAKGQPREPQVCTLPPSRDELTKNQVSLSCAVKGFYPSDIAVEWESNGQPENNYKTTPPVLDSDGSFFLVSKLTVDKSRWQQGNVFSCSVMHEALHNHYTQKSLSLSPGK

SEQ ID NO: 53 - protein, 178 aa, synthetic construct
  source 1..178: note = RO7122290
REGPELSPDDPAGLLDLRQGMFAQLVAQNVLLIDGPLSWYSDPGLAGVSLTGGLSYKEDTKELVVAKAGVYYVFFQLELRRVVAGEGSGSVSLALHLQPLRSAAGAAALALTVDLPPASSEARNSAFGFQGRLLHLSAGQRLGVHLHTEARARHAWQLTQGATVLGLFRVTPEIPAGL

SEQ ID NO: 54 - protein, 215 aa, synthetic construct
  source 1..215: note = RO7122290
EIVLTQSPGTLSLSPGERATLSCRASQSVTSSYLAWYQQKPGQAPRLLINVGSRRATGIPDRFSGSGSGTDFTLTISRLEPEDFAVYYCQQGIMLPPTFGQGTKVEIKRTVAAPSVFIFPPSDEQLKSGTASVVCLLNNFYPREAKVQWKVDNALQSGNSQESVTEQDSKDSTYSLSSTLTLSKADYEKHKVYACEVTHQGLSSPVTKSFNRGEC

SEQ ID NO: 55 - protein, 676 aa, synthetic construct
  source 1..676: note = RO7300490
QVQLVQSGAEVKKPGASVKVSCKASGYSFTGYYIHWVRQAPGQSLEWMGRVIPNAGGTSYNQKFKGRVTLTVDKSISTAYMELSRLRSDDTAVYYCAREGIYWWGQGTTVTVSSASTKGPSVFPLAPSSKSTSGGTAALGCLVEDYFPEPVTVSWNSGALTSGVHTFPAVLQSSGLYSLSSVVTVPSSSLGTQTYICNVNHKPSNTKVDEKVEPKSCDKTHTCPPCPAPEAAGGPSVFLFPPKPKDTLMISRTPEVTCVVVDVSHEDPEVKFNWYVDGVEVHNAKTKPREEQYNSTYRVVSVLTVLHQDWLNGKEYKCKVSNKALGAPIEKTISKAKGQPREPQVYTLPPCRDELTKNQVSLWCLVKGFYPSDIAVEWESNGQPENNYKTTPPVLDSDGSFFLYSKLTVDKSRWQQGNVFSCSVMHEALHNHYTQKSLSLSPGGGGGSGGGGSGGGGSGGGGSEIVLTQSPGTLSLSPGERATLSCRASQSVSRSYLAWYQQKPGQAPRLLIIGASTRATGIPDRFSGSGSGTDFTLTISRLEPEDFAVYYCQQGQVIPPTFGQGTKVEIKSSASTKGPSVFPLAPSSKSTSGGTAALGCLVKDYFPEPVTVSWNSGALTSGVHTFPAVLQSSGLYSLSSVVTVPSSSLGTQTYICNVNHKPSNTKVDKKVEPKSC

SEQ ID NO: 56 - protein, 223 aa, synthetic construct
  source 1..223: note = RO7300490
EVQLLESGGGLVQPGGSLRLSCAASGFTFSSHAMSWVRQAPGKGLEWVSAIWASGEQYYADSVKGRFTISRDNSKNTLYLQMNSLRAEDTAVYYCAKGWLGNFDYWGQGTLVTVSSASVAAPSVFIFPPSDEQLKSGTASVVCLLNNFYPREAKVQWKVDNALQSGNSQESVTEQDSKDSTYSLSSTLTLSKADYEKHKVYACEVTHQGLSSPVTKSFNRGEC

SEQ ID NO: 57 - protein, 443 aa, synthetic construct
  source 1..443: note = RO7300490
QVQLVQSGAEVKKPGASVKVSCKASGYSFTGYYIHWVRQAPGQSLEWMGRVIPNAGGTSYNQKFKGRVTLTVDKSISTAYMELSRLRSDDTAVYYCAREGIYWWGQGTTVTVSSASTKGPSVFPLAPSSKSTSGGTAALGCLVEDYFPEPVTVSWNSGALTSGVHTFPAVLQSSGLYSLSSVVTVPSSSLGTQTYICNVNHKPSNTKVDEKVEPKSCDKTHTCPPCPAPEAAGGPSVFLFPPKPKDTLMISRTPEVTCVVVDVSHEDPEVKFNWYVDGVEVHNAKTKPREEQYNSTYRVVSVLTVLHQDWLNGKEYKCKVSNKALGAPIEKTISKAKGQPREPQVCTLPPSRDELTKNQVSLSCAVKGFYPSDIAVEWESNGQPENNYKTTPPVLDSDGSFFLVSKLTVDKSRWQQGNVFSCSVMHEALHNHYTQKSLSLSPG

SEQ ID NO: 58 - protein, 219 aa, synthetic construct
  source 1..219: note = RO7300490
DIVMTQTPLSLSVTPGQPASISCRSSQSLVHSNGNTFLHWYLQKPGQSPQLLIYTVSNRFSGVPDRFSGSGSGTDFTLKISRVEAEDVGVYFCSQTTHVPWTFGGGTKVEIKRTVAAPSVFIFPPSDRKLKSGTASVVCLLNNFYPREAKVQWKVDNALQSGNSQESVTEQDSKDSTYSLSSTLTLSKADYEKHKVYACEVTHQGLSSPVTKSFNRGEC

SEQ ID NO: 59 - protein, 582 aa, synthetic construct
  source 1..582: note = Ab10-A12V2-2
QVQLQQSGVEVKKPGASVTVSCRASGYSFADHFIHWVRQAPGQGFQWMGWINPNRGVTHHAQDFQGRVAMTRDMSTDTVYMELTSLRSDDTAVYYCARDASLTARPYYFYGFDVWGQGTLVTVSSASTKGPSVFPLAPSSKSTSGGTAALGCLVKDYFPEPVTVSWNSGALTSGVHTFPAVLQSSGLYSLSSVVTVPSSSLGTQTYICNVNHKPSNTKVDKKVEPKSCDKTHTCPPCPAPEAAGGPSVFLFPPKPKDTLMISRTPEVTCVVVDVSHEDPEVKFNWYVDGVEVHNAKTKPREEQYNSTYRVVSVLTVLHQDWLNGKEYKCKVSNKALPAPIEKTISKAKGQPREPQVYTLPPSRDELTKNQVSLTCLVKGFYPSDIAVEWESNGQPENNYKTTPPVLDSDGSFFLYSKLTVDKSRWQQGNVFSCSVMHEALHNHYTQKSLSLSPGKGGGGSGGGGSEVQLVESGGGLVQPGGSLRLSCAASGFTFSNYGMKWVRQAPGKGLEWVSTILSQGGSTYYADSVKGRFTISRDNAKNSLYLQMNSLRAEDTALYYCLRVDWSDYSPRGQGTQVTVSS

SEQ ID NO: 60 - protein, 214 aa, synthetic construct; identical to SEQ ID NO: 10
  source 1..214: note = Ab10-A12V2-2

SEQ ID NO: 61 - protein, 757 aa, synthetic construct
  source 1..757: note = MP0310
GSDLGKKLLEAARAGQDDEVRELLKAGADVNAKDYFSHTPLHLAARNGHLKIVEVLLKAGADVNAKDFAGKTPLHLAAADGHLEIVEVLLKAGADVNAQDIFGKTPADIAADAGHEDIAEVLQKAAGSPTPTPTTPTPTPTTPTPTPTGSDLGKKLLEAARAGQDDEVRELLKAGADVNAKDVLGWTPLHLAAFEGHLEIVEVLLKAGADVNAKDKKGWTPLQLAARTGHLEIVEVLLKAGADVNAKDHIGATPLHLAAWQGHPEIVEVLLKAGADVNAQDKSGKTPADLAADAGHEDIAEVLQKAAGSPTPTPTTPTPTPTTPTPTPTGSDLGQKLLKAAQEGQDDEVRELLKAGADVNAKDLRGITPLHVAAWQGHLEIVEVLLKAGADVNAKDSKGETPLHLAAFRGHLEIVEVLLKAGADVNAQDQQGETPADLAALAGHVDIAEVLQKAAGSPTPTPTTPTPTPTTPTPTPTGSDLGQKLLKAAQEGQDDEVRELLKAGADVNAKDLRGITPLHVAAWQGHLEIVEVLLKAGADVNAKDSKGETPLHLAAFRGHLEIVEVLLKAGADVNAQDQQGETPADLAALAGHVDIAEVLQKAAGSPTPTPTTPTPTPTTPTPTPTGSDLGKKLLEAARAGQDDEVRELLKAGADVNAKDYFSHTPLHLAARNGHLKIVEVLLKAGADVNAKDFAGKTPLHLAAADGHLEIVEVLLKAGADVNAQDIFGKTPADIAADAGHEDIAEVLQKAAHHHHHH

SEQ ID NO: 62 - protein, 452 aa, synthetic construct
  source 1..452: note = BNT312
EVQLVQSGAEVKKPGASVKVSCKTSGYTFTEYIMHWVRQAPGQGLEWMGGIIPNNGGTSYNQKFQGRVTMTVDKSTSTGYMELSSLRSEDTAVYYCTRREVYGRNYYALDYWGQGTLVTVSSASTKGPSVFPLAPSSKSTSGGTAALGCLVKDYFPEPVTVSWNSGALTSGVHTFPAVLQSSGLYSLSSVVTVPSSSLGTQTYICNVNHKPSNTKVDKRVEPKSCDKTHTCPPCPAPEFEGGPSVFLFPPKPKDTLMISRTPEVTCVVVAVSHEDPEVKFNWYVDGVEVHNAKTKPREEQYNSTYRVVSVLTVLHQDWLNGKEYKCKVSNKALPAPIEKTISKAKGQPREPQVYTLPPSREEMTKNQVSLTCLVKGFYPSDIAVEWESNGQPENNYKTTPPVLDSDGSFLLYSKLTVDKSRWQQGNVFSCSVMHEALHNHYTQKSLSLSPGK

SEQ ID NO: 63 - protein, 214 aa, synthetic construct
  source 1..214: note = BNT312
DIQMTQSPSSLSASVGDRVTITCSASQGINNYLNWYQQKPGKAVKLLIYYTSSLHSGVPSRFSGSGSGTDYTFTISSLQPEDIATYYCQQYSNLPYTFGGGTKVEIKRTVAAPSVFIFPPSDEQLKSGTASVVCLLNNFYPREAKVQWKVDNALQSGNSQESVTEQDSKDSTYSLSSTLTLSKADYEKHKVYACEVTHQGLSSPVTKSFNRGEC

SEQ ID NO: 64 - protein, 447 aa, synthetic construct
  source 1..447: note = BNT312
EVQLVESGGGLVQPGRSLRLSCTASGFSLNDYWMSWVRQAPGKGLEWVGYIDVGGSLYYAASVKGRFTISRDDSKSIAYLQMNSLKTEDTAVYYCARGGLTYGFDLWGQGTLVTVSSASTKGPSVFPLAPSSKSTSGGTAALGCLVKDYFPEPVTVSWNSGALTSGVHTFPAVLQSSGLYSLSSVVTVPSSSLGTQTYICNVNHKPSNTKVDKRVEPKSCDKTHTCPPCPAPEFEGGPSVFLFPPKPKDTLMISRTPEVTCVVVAVSHEDPEVKFNWYVDGVEVHNAKTKPREEQYNSTYRVVSVLTVLHQDWLNGKEYKCKVSNKALPAPIEKTISKAKGQPREPQVYTLPPSREEMTKNQVSLTCLVKGFYPSDIAVEWESNGQPENNYKTTPPVLDSDGSFFLYSRLTVDKSRWQQGNVFSCSVMHEALHNHYTQKSLSLSPGK

SEQ ID NO: 65 - protein, 217 aa, synthetic construct
  source 1..217: note = BNT312
DIVMTQSPSSLSASVGDRVTITCQASEDISSYLAWYQQKPGKAPKRLIYGASDLASGVPSRFSASGSGTDYTFTISSLQPEDIATYYCHYYATISGLGVAFGGGTKVEIKRTVAAPSVFIFPPSDEQLKSGTASVVCLLNNFYPREAKVQWKVDNALQSGNSQESVTEQDSKDSTYSLSSTLTLSKADYEKHKVYACEVTHQGLSSPVTKSFNRGEC

SEQ ID NO: 66 - protein, 223 aa, synthetic construct
  source 1..223: note = Fab
QVQLQQSGVEVKKPGASVTVSCRASGYSFADHFIHWVRQAPGQGFQWMGWINPNRGVTHHAQDFQGRVAMTRDMSTDTVYMELTSLRSDDTAVYYCARDASLTARPYYFYGFDVWGQGTLVTVSSASTKGPSVFPLAPSSKSTSGGTAALGCLVKDYFPEPVTVSWNSGALTSGVHTFPAVLQSSGLYSLSSVVTVPSSSLGTQTYICNVNHKPSNTKVDKKV

SEQ ID NO: 67 - protein, 214 aa, synthetic construct; identical to SEQ ID NO: 10
  source 1..214: note = Fab

SEQ ID NO: 68 - protein, 4 aa, synthetic construct
  source 1..4: note = c-terminal; note (original language) = C-terminal
TVSS

SEQ ID NO: 69 - protein, 5 aa, synthetic construct
  source 1..5: note = c-terminal; note (original language) = C-terminal
TVSAA

SEQ ID NO: 70 - protein, 7 aa, synthetic construct
  source 1..7: note = c-terminal; note (original language) = C-terminal
TLVTVSS

SEQ ID NO: 71 - protein, 7 aa, synthetic construct
  source 1..7: note = c-terminal; note (original language) = C-terminal
TQVTVSS

SEQ ID NO: 72 - protein, 6 aa, synthetic construct
  source 1..6: note = linker; note (original language) = Linker
GGNGTH

SEQ ID NO: 73 - protein, 6 aa, synthetic construct
  source 1..6: note = linker; note (original language) = Linker
YGNGTH

SEQ ID NO: 74 - protein, 6 aa, synthetic construct
  source 1..6: note = linker; note (original language) = Linker
EPKSSH

SEQ ID NO: 75 - protein, 5 aa, synthetic construct
  source 1..5: note = linker; note (original language) = Linker
GGGGS

SEQ ID NO: 76 - protein, 10 aa, synthetic construct
  source 1..10: note = linker; note (original language) = Linker
GGGGSGGGGS

SEQ ID NO: 77 - protein, 15 aa, synthetic construct
  source 1..15: note = linker; note (original language) = Linker
GGGGSGGGGSGGGGS

SEQ ID NO: 78 - protein, 20 aa, synthetic construct
  source 1..20: note = linker; note (original language) = Linker
GGGGSGGGGSGGGGSGGGGS

SEQ ID NO: 79 - protein, 25 aa, synthetic construct
  source 1..25: note = linker; note (original language) = Linker
GGGGSGGGGSGGGGSGGGGSGGGGS

SEQ ID NO: 80 - protein, 4 aa, synthetic construct
  source 1..4: note = linker; note (original language) = Linker
ASGS